European Patent Specification EP 3 167 396 B1, published January 17, 2024. Title: IMMUNE RECOGNITION MOTIFS. Applicant: IOGENETICS, LLC. The sequence listing filed with the application follows.

SEQUENCE LISTING (488 sequences)

SEQ ID NO: 1 - protein, 15 aa, artificial sequence
  any amino acid
FAMERNAGSGIIISD

SEQ ID NO: 2 - protein, 5 aa, artificial sequence
  any amino acid
RNGGI

SEQ ID NO: 3 - protein, 5 aa, artificial sequence
  any amino acid
MNGGI

SEQ ID NO: 4 - protein, 15 aa, artificial sequence
  any amino acid
AMERNAGSGIIISDT

SEQ ID NO: 5 - protein, 5 aa, artificial sequence
  any amino acid
NASII

SEQ ID NO: 6 - protein, 5 aa, artificial sequence
  any amino acid
EASII

SEQ ID NO: 7 - protein, 15 aa, artificial sequence
  any amino acid
MERNAGSGIIISDTP

SEQ ID NO: 8 - protein, 5 aa, artificial sequence
  any amino acid
AGGII

SEQ ID NO: 9 - protein, 5 aa, artificial sequence
  any amino acid
RGGII

SEQ ID NO: 10 - protein, 15 aa, artificial sequence
  any amino acid
ERNAGSGIIISDTPV

SEQ ID NO: 11 - protein, 5 aa, artificial sequence
  any amino acid
GSIIS

SEQ ID NO: 12 - protein, 5 aa, artificial sequence
  any amino acid
NSIIS

SEQ ID NO: 13 - protein, 15 aa, artificial sequence
  any amino acid
RNAGSGIIISDTPVH

SEQ ID NO: 14 - protein, 5 aa, artificial sequence
  any amino acid
SGISD

SEQ ID NO: 15 - protein, 5 aa, artificial sequence
  any amino acid
AGISD

SEQ ID NO: 16 - protein, 5 aa, artificial sequence
  any amino acid
VPGLV

SEQ ID NO: 17 - protein, 5 aa, artificial sequence
  any amino acid
VPGIV

SEQ ID NO: 18 - protein, 5 aa, artificial sequence
  any amino acid
TGIGS

SEQ ID NO: 19 - protein, 5 aa, artificial sequence
  any amino acid
TGIDS

SEQ ID NO: 20 - protein, 5 aa, artificial sequence
  any amino acid
SLSVA

SEQ ID NO: 21 - protein, 5 aa, artificial sequence
  any amino acid
SLSIA

SEQ ID NO: 22 - protein, 5 aa, artificial sequence
  any amino acid
GVTTN

SEQ ID NO: 23 - protein, 5 aa, artificial sequence
  any amino acid
GVTTD

SEQ ID NO: 24 - protein, 5 aa, artificial sequence
  any amino acid
TVSST

SEQ ID NO: 25 - protein, 5 aa, artificial sequence
  any amino acid
TVSTT

SEQ ID NO: 26 - protein, 5 aa, artificial sequence
  any amino acid
LSYIS

SEQ ID NO: 27 - protein, 5 aa, artificial sequence
  any amino acid
LSYIF

SEQ ID NO: 28 - protein, 5 aa, artificial sequence
  any amino acid
STATL

SEQ ID NO: 29 - protein, 5 aa, artificial sequence
  any amino acid
RTATL

SEQ ID NO: 30 - protein, 5 aa, artificial sequence
  any amino acid
GSSTG

SEQ ID NO: 31 - protein, 5 aa, artificial sequence
  any amino acid
SSSTG

SEQ ID NO: 32 - protein, 5 aa, artificial sequence
  any amino acid
SLSIA

SEQ ID NO: 33 - protein, 5 aa, artificial sequence
  any amino acid
TGIDS

SEQ ID NO: 34 - protein, 5 aa, artificial sequence
  any amino acid
RSTAY

SEQ ID NO: 35 - protein, 15 aa, artificial sequence
  any amino acid
DESKSLKSQIAEAKI

SEQ ID NO: 36 - protein, 15 aa, artificial sequence
  any amino acid
APGISLPSLIAGQPG

SEQ ID NO: 37 - protein, 15 aa, artificial sequence
  any amino acid
WIIQSLASAIAYLHN

SEQ ID NO: 38 - protein, 15 aa, artificial sequence
  any amino acid
VTLSSLSSAIAKHES

SEQ ID NO: 39 - protein, 15 aa, artificial sequence
  any amino acid
GPPSSLMSEIADLTF

SEQ ID NO: 40 - protein, 15 aa, artificial sequence
  any amino acid
SLSLSLPSTIAAPHP

SEQ ID NO: 41 - protein, 15 aa, artificial sequence
  any amino acid
LFPHSLLSVIANFIP

SEQ ID NO: 42 - protein, 15 aa, artificial sequence
  any amino acid
APGISLPSLIAGQPG

SEQ ID NO: 43 - protein, 15 aa, artificial sequence
  any amino acid
LFPHSLLSVIANFIP

SEQ ID NO: 44 - protein, 15 aa, artificial sequence
  any amino acid
WIIQSLASAIAYLHN

SEQ ID NO: 45 - protein, 15 aa, artificial sequence
  any amino acid
ALEASLISQIADSLK

SEQ ID NO: 46 - protein, 15 aa, artificial sequence
  any amino acid
VNLFSLGSAIAYSAY

SEQ ID NO: 47 - protein, 15 aa, artificial sequence
  any amino acid
NDTVSLASSIATQPE

SEQ ID NO: 48 - protein, 15 aa, artificial sequence
  any amino acid
GPPSSLMSEIADLTF

SEQ ID NO: 49 - protein, 15 aa, artificial sequence
  any amino acid
LGEQSLQSRIAALTV

SEQ ID NO: 50 - protein, 15 aa, artificial sequence
  any amino acid
SSRTSLVSTIAGILS

SEQ ID NO: 51 - protein, 15 aa, artificial sequence
  any amino acid
PQITSLPSNIALSPT

SEQ ID NO: 52 - protein, 15 aa, artificial sequence
  any amino acid
TVSYSLLSGIALNDR

SEQ ID NO: 53 - protein, 15 aa, artificial sequence
  any amino acid
DESKSLKSQIAEAKI

SEQ ID NO: 54 - protein, 15 aa, artificial sequence
  any amino acid
GIISSLFSLIAGIIL

SEQ ID NO: 55 - protein, 15 aa, artificial sequence
  any amino acid
APGISLPSLIAGQPG

SEQ ID NO: 56 - protein, 15 aa, artificial sequence
  any amino acid
SSRTSLVSTIAGILS

SEQ ID NO: 57 - protein, 15 aa, artificial sequence
  any amino acid
VNAISLTSGIAKGLN

SEQ ID NO: 58 - protein, 15 aa, artificial sequence
  any amino acid
ECSGSLGSGIAEVCL

SEQ ID NO: 59 - protein, 15 aa, artificial sequence
  any amino acid
SVFSSLSSPIAAPIS

SEQ ID NO: 60 - protein, 15 aa, artificial sequence
  any amino acid
DESKSLKSQIAEAKI

SEQ ID NO: 61 - protein, 15 aa, artificial sequence
  any amino acid
SLNVSLESLIANLCA

SEQ ID NO: 62 - protein, 15 aa, artificial sequence
  any amino acid
ERAASLFSAIAKFKA

SEQ ID NO: 63 - protein, 15 aa, artificial sequence
  any amino acid
DESKSLKSQIAEAKI

SEQ ID NO: 64 - protein, 15 aa, artificial sequence
  any amino acid
VTLSSLSSAIAKHES

SEQ ID NO: 65 - protein, 15 aa, artificial sequence
  any amino acid
SLSLSLPSTIAAPHP

SEQ ID NO: 66 - protein, 15 aa, artificial sequence
  any amino acid
NDTVSLASSIATQPE

SEQ ID NO: 67 - protein, 15 aa, artificial sequence
  any amino acid
PQITSLPSNIALSPT

SEQ ID NO: 68 - protein, 15 aa, artificial sequence
  any amino acid
WIIQSLASAIAYLHN

SEQ ID NO: 69 - protein, 15 aa, artificial sequence
  any amino acid
WRGLSLDSPIAVLLT

SEQ ID NO: 70 - protein, 15 aa, artificial sequence
  any amino acid
GPPSSLMSEIADLTF

SEQ ID NO: 71 - protein, 15 aa, artificial sequence
  any amino acid
IREISLDSCIAQSYF

SEQ ID NO: 72 - protein, 15 aa, artificial sequence
  any amino acid
LFPHSLLSVIANFIP

SEQ ID NO: 73 - protein, 15 aa, artificial sequence
  any amino acid
VPIYSLDSWIALKYP

SEQ ID NO: 74 - protein, 15 aa, artificial sequence
  any amino acid
VNLFSLGSAIAYSAY

SEQ ID NO: 75 - protein, 15 aa, artificial sequence
  any amino acid
IVAVSLVSLIANALG

SEQ ID NO: 76 - protein, 15 aa, artificial sequence
  any amino acid
LLLSSLTSPIAENSP

SEQ ID NO: 77 - protein, 15 aa, artificial sequence
  any amino acid
GPSSSLMSEIADLTY

SEQ ID NO: 78 - protein, 15 aa, artificial sequence
  any amino acid
VVYKVPKGKIVPNLN

SEQ ID NO: 79 - protein, 15 aa, artificial sequence
  any amino acid
LLHEVPTGEIVVRLD

SEQ ID NO: 80 - protein, 15 aa, artificial sequence
  any amino acid
NWGAVPFGKIVGKFP

SEQ ID NO: 81 - protein, 15 aa, artificial sequence
  any amino acid
CVPSVPVGPIVLTSA

SEQ ID NO: 82 - protein, 15 aa, artificial sequence
  any amino acid
FRTKVPEGLIVFAAS

SEQ ID NO: 83 - protein, 15 aa, artificial sequence
  any amino acid
PIEDVPCGNIVGLVG

SEQ ID NO: 84 - protein, 15 aa, artificial sequence
  any amino acid
LLHEVPTGEIVVRLD

SEQ ID NO: 85 - protein, 15 aa, artificial sequence
  any amino acid
VVYKVPKGKIVPNLN

SEQ ID NO: 86 - protein, 15 aa, artificial sequence
  any amino acid
NDLDVPVGHIVHTGM

SEQ ID NO: 87 - protein, 15 aa, artificial sequence
  any amino acid
LEDRVPSGLIVDYHN

SEQ ID NO: 88 - protein, 15 aa, artificial sequence
  any amino acid
QEASVPKGRIVPRGI

SEQ ID NO: 89 - protein, 15 aa, artificial sequence
  any amino acid
GPVHVPLGHIVANEK

SEQ ID NO: 90 - protein, 15 aa, artificial sequence
  any amino acid
NWGAVPFGKIVGKFP

SEQ ID NO: 91 - protein, 15 aa, artificial sequence
  any amino acid
VSWDVPEGNIVIGYS

SEQ ID NO: 92 - protein, 9 aa, artificial sequence
  any amino acid
EEAAGIGIL

SEQ ID NO: 93 - protein, 9 aa, artificial sequence
  any amino acid
EAAGIGILT

SEQ ID NO: 94 - protein, 9 aa, artificial sequence
  any amino acid
AAGIGILTV

SEQ ID NO: 95 - protein, 9 aa, artificial sequence
  any amino acid
AGIGILTVI

SEQ ID NO: 96 - protein, 9 aa, artificial sequence
  any amino acid
GIGILTVIL

SEQ ID NO: 97 - protein, 9 aa, artificial sequence
  any amino acid
IGILTVILG

SEQ ID NO: 98 - protein, 9 aa, artificial sequence
  any amino acid
GILTVILGV

SEQ ID NO: 99 - protein, 9 aa, artificial sequence
  any amino acid
ILTVILGVL

SEQ ID NO: 100 - protein, 9 aa, artificial sequence
  any amino acid
LTVILGVLL

SEQ ID NO: 101 - protein, 9 aa, artificial sequence
  any amino acid
TVILGVLLL

SEQ ID NO: 102 - protein, 9 aa, artificial sequence
  any amino acid
VILGVLLLI

SEQ ID NO: 103 - protein, 9 aa, artificial sequence
  any amino acid
ILGVLLLIG

SEQ ID NO: 104 - protein, 9 aa, artificial sequence
  any amino acid
LGVLLLIGC

SEQ ID NO: 105 - protein, 9 aa, artificial sequence
  any amino acid
GVLLLIGCW

SEQ ID NO: 106 - protein, 9 aa, artificial sequence
  any amino acid
VLLLIGCWY

SEQ ID NO: 107 - protein, 9 aa, artificial sequence
  any amino acid
LLLIGCWYC

SEQ ID NO: 108 - protein, 9 aa, artificial sequence
  any amino acid
LLIGCWYCR

SEQ ID NO: 109 - protein, 9 aa, artificial sequence
  any amino acid
LIGCWYCRR

SEQ ID NO: 110 - protein, 9 aa, artificial sequence
  any amino acid
IGCWYCRRR

SEQ ID NO: 111 - protein, 9 aa, artificial sequence
  any amino acid
GCWYCRRRN

SEQ ID NO: 112 - protein, 9 aa, artificial sequence
  any amino acid
CWYCRRRNG

SEQ ID NO: 113 - protein, 9 aa, artificial sequence
  any amino acid
WYCRRRNGY

SEQ ID NO: 114 - protein, 9 aa, artificial sequence
  any amino acid
YCRRRNGYR

SEQ ID NO: 115 - protein, 9 aa, artificial sequence
  any amino acid
CRRRNGYRA

SEQ ID NO: 116 - protein, 9 aa, artificial sequence
  any amino acid
RRRNGYRAL

SEQ ID NO: 117 - protein, 9 aa, artificial sequence
  any amino acid
RRNGYRALM

SEQ ID NO: 118 - protein, 8 aa, artificial sequence
  any amino acid
PFSVSVSQ

SEQ ID NO: 119 - protein, 8 aa, artificial sequence
  any amino acid
  misc_feature (1)..(2): Xaa can be any naturally occurring amino acid
  misc_feature (8)..(8): Xaa can be any naturally occurring amino acid
XXSVSVSX

SEQ ID NO: 120 - protein, 8 aa, artificial sequence
  any amino acid
TTPGQAPT

SEQ ID NO: 121 - protein, 8 aa, artificial sequence
  any amino acid
  misc_feature (1)..(2): Xaa can be any naturally occurring amino acid
  misc_feature (8)..(8): Xaa can be any naturally occurring amino acid
XXPGQAPX

SEQ ID NO: 122 - protein, 15 aa, artificial sequence
  any amino acid
LGVLLLIGCWYCRRR

SEQ ID NO: 123 - protein, 7 aa, artificial sequence
  any amino acid
  misc_feature (3)..(3): Xaa can be any naturally occurring amino acid
  misc_feature (5)..(5): Xaa can be any naturally occurring amino acid
LLXGXWY

SEQ ID NO: 124 - protein, 9 aa, artificial sequence
  any amino acid
  misc_feature (2)..(3): Xaa can be any naturally occurring amino acid
  misc_feature (5)..(5): Xaa can be any naturally occurring amino acid
  misc_feature (7)..(7): Xaa can be any naturally occurring amino acid
VXXLXGXWY

SEQ ID NO: 125 - protein, 15 aa, artificial sequence
  any amino acid
SSSSPLVLGTLEEVP

SEQ ID NO: 126 - protein, 9 aa, artificial sequence
  any amino acid
  misc_feature (2)..(3): Xaa can be any naturally occurring amino acid
  misc_feature (5)..(5): Xaa can be any naturally occurring amino acid
  misc_feature (7)..(7): Xaa can be any naturally occurring amino acid
SXXLXLXTL

SEQ ID NO: 127 - protein, 15 aa, artificial sequence
  any amino acid
SSSPLVLGTLEEVPT

SEQ ID NO: 128 - protein, 7 aa, artificial sequence
  any amino acid
  misc_feature (3)..(3): Xaa can be any naturally occurring amino acid
  misc_feature (5)..(5): Xaa can be any naturally occurring amino acid
LVXGXLE

SEQ ID NO: 129 - protein, 15 aa, artificial sequence
  any amino acid
SPLVLGTLEEVPTAG

SEQ ID NO: 130 - protein, 7 aa, artificial sequence
  any amino acid
  misc_feature (3)..(3): Xaa can be any naturally occurring amino acid
  misc_feature (5)..(5): Xaa can be any naturally occurring amino acid
LGXLXEV

SEQ ID NO: 131 - protein, 15 aa, artificial sequence
  any amino acid
TGFLIIVLVMIAMEG

SEQ ID NO: 132 - protein, 7 aa, artificial sequence
  any amino acid
  misc_feature (3)..(3): Xaa can be any naturally occurring amino acid
  misc_feature (5)..(5): Xaa can be any naturally occurring amino acid
IIXLXMI

SEQ ID NO: 133 - protein, 15 aa, artificial sequence
  any amino acid
GFLIIVLVMIAMEGG

SEQ ID NO: 134 - protein, 8 aa, artificial sequence
  any amino acid
  misc_feature (2)..(2): Xaa can be any naturally occurring amino acid
  misc_feature (4)..(4): Xaa can be any naturally occurring amino acid
  misc_feature (6)..(6): Xaa can be any naturally occurring amino acid
LXVXVXIA

SEQ ID NO: 135 - protein, 15 aa, artificial sequence
  any amino acid
LDVMASQKRPSQRHG

SEQ ID NO: 136 - protein, 7 aa, artificial sequence
  any amino acid
  misc_feature (3)..(3): Xaa can be any naturally occurring amino acid
  misc_feature (5)..(5): Xaa can be any naturally occurring amino acid
ASXKXPS

SEQ ID NO: 137 - protein, 15 aa, artificial sequence
  any amino acid
SQGKGRGLSLSRFSW

SEQ ID NO: 138 - protein, 7 aa, artificial sequence
  any amino acid
  misc_feature (3)..(3): Xaa can be any naturally occurring amino acid
  misc_feature (5)..(5): Xaa can be any naturally occurring amino acid
GRXLXLS

SEQ ID NO: 139 - protein, 15 aa, artificial sequence
  any amino acid
TLSKIFKLGGRDSRS

SEQ ID NO: 140 - protein, 7 aa, artificial sequence
  any amino acid
  misc_feature (3)..(3): Xaa can be any naturally occurring amino acid
  misc_feature (5)..(5): Xaa can be any naturally occurring amino acid
IFXLXGR

SEQ ID NO: 141 - protein, 5 aa, artificial sequence
  any amino acid
NQLGT

SEQ ID NO: 142 - protein, 5 aa, artificial sequence
  any amino acid
VCRYR

SEQ ID NO: 143 - protein, 5 aa, artificial sequence
  any amino acid
QQGEV

SEQ ID NO: 144 - protein, 5 aa, artificial sequence
  any amino acid
RLVSS

SEQ ID NO: 145 - protein, 5 aa, artificial sequence
  any amino acid
LLMSL

SEQ ID NO: 146 - protein, 5 aa, artificial sequence
  any amino acid
LYQPD

SEQ ID NO: 147 - protein, 5 aa, artificial sequence
  any amino acid
LLMSL

SEQ ID NO: 148 - protein, 5 aa, artificial sequence
  any amino acid
PETLY

SEQ ID NO: 149 - protein, 5 aa, artificial sequence
  any amino acid
LETLY

SEQ ID NO: 150 - protein, 5 aa, artificial sequence
  any amino acid
SKKTL

SEQ ID NO: 151 - protein, 5 aa, artificial sequence
  any amino acid
YCSDS

SEQ ID NO: 152 - protein, 5 aa, artificial sequence
  any amino acid
TYCTT

SEQ ID NO: 153 - protein, 5 aa, artificial sequence
  any amino acid
PEFLY

SEQ ID NO: 154 - protein, 5 aa, artificial sequence
  any amino acid
LEFLY

SEQ ID NO: 155 - protein, 5 aa, artificial sequence
  any amino acid
KEGTL

SEQ ID NO: 156 - protein, 5 aa, artificial sequence
  any amino acid
KSSKN

SEQ ID NO: 157 - protein, 5 aa, artificial sequence
  any amino acid
LTRLQ

SEQ ID NO: 158 - protein, 5 aa, artificial sequence
  any amino acid
RGCAR

SEQ ID NO: 159 - protein, 5 aa, artificial sequence
  any amino acid
IFKEL

SEQ ID NO: 160 - protein, 5 aa, artificial sequence
  any amino acid
SGGTV

SEQ ID NO: 161 - protein, 5 aa, artificial sequence
  any amino acid
TCVGA

SEQ ID NO: 162 - protein, 5 aa, artificial sequence
  any amino acid
LVRRS

SEQ ID NO: 163 - protein, 5 aa, artificial sequence
  any amino acid
YSSYG

SEQ ID NO: 164 - protein, 5 aa, artificial sequence
  any amino acid
SVGTL

SEQ ID NO: 165 - protein, 5 aa, artificial sequence
  any amino acid
KKSLY

SEQ ID NO: 166 - protein, 5 aa, artificial sequence
  any amino acid
TRTAT

SEQ ID NO: 167 - protein, 5 aa, artificial sequence
  any amino acid
VYGAS

SEQ ID NO: 168 - protein, 5 aa, artificial sequence
  any amino acid
SRYYY

SEQ ID NO: 169 - protein, 5 aa, artificial sequence
  any amino acid
LRLSC

SEQ ID NO: 170 - protein, 5 aa, artificial sequence
  any amino acid
RLSCV

SEQ ID NO: 171 - protein, 5 aa, artificial sequence
  any amino acid
LLLLS

SEQ ID NO: 172 - protein, 5 aa, artificial sequence
  any amino acid
YTSLQ

SEQ ID NO: 173 - protein, 5 aa, artificial sequence
  any amino acid
LRLSC

SEQ ID NO: 174 - protein, 5 aa, artificial sequence
  any amino acid
RLSCV

SEQ ID NO: 175 - protein, 5 aa, artificial sequence
  any amino acid
RNNWP

SEQ ID NO: 176 - protein, 5 aa, artificial sequence
  any amino acid
IETVY

SEQ ID NO: 177 - protein, 5 aa, artificial sequence
  any amino acid
RQRQR

SEQ ID NO: 178 - protein, 5 aa, artificial sequence
  any amino acid
KFVRD

SEQ ID NO: 179 - protein, 5 aa, artificial sequence
  any amino acid
SVGTL

SEQ ID NO: 180 - protein, 5 aa, artificial sequence
  any amino acid
LTRTQ

SEQ ID NO: 181 - protein, 5 aa, artificial sequence
  any amino acid
YSDSV

SEQ ID NO: 182 - protein, 5 aa, artificial sequence
  any amino acid
YYSDS

SEQ ID NO: 183 - protein, 5 aa, artificial sequence
  any amino acid
AGSYT

SEQ ID NO: 184 - protein, 5 aa, artificial sequence
  any amino acid
LETVY

SEQ ID NO: 185 - protein, 5 aa, artificial sequence
  any amino acid
SVGTL

SEQ ID NO: 186 - protein, 5 aa, artificial sequence
  any amino acid
DSTYC

SEQ ID NO: 187 - protein, 5 aa, artificial sequence
  any amino acid
QPKPQ

SEQ ID NO: 188 - protein, 5 aa, artificial sequence
  any amino acid
TDTVY

SEQ ID NO: 189 - protein, 5 aa, artificial sequence
  any amino acid
ADTVY

SEQ ID NO: 190 - protein, 5 aa, artificial sequence
  any amino acid
YCQLQ

SEQ ID NO: 191 - protein, 5 aa, artificial sequence
  any amino acid
EEIEI

SEQ ID NO: 192 - protein, 5 aa, artificial sequence
  any amino acid
HSRTG

SEQ ID NO: 193 - protein, 5 aa, artificial sequence
  any amino acid
TLMTL

SEQ ID NO: 194 - protein, 5 aa, artificial sequence
  any amino acid
ASSTS

SEQ ID NO: 195 - protein, 5 aa, artificial sequence
  any amino acid
DATAT

SEQ ID NO: 196 - protein, 5 aa, artificial sequence
  any amino acid
VRTST

SEQ ID NO: 197 - protein, 5 aa, artificial sequence
  any amino acid
SLLCA

SEQ ID NO: 198 - protein, 5 aa, artificial sequence
  any amino acid
EGIYR

SEQ ID NO: 199 - protein, 5 aa, artificial sequence
  any amino acid
GDSLR

SEQ ID NO: 200 - protein, 5 aa, artificial sequence
  any amino acid
SRDTL

SEQ ID NO: 201 - protein, 5 aa, artificial sequence
  any amino acid
PETLY

SEQ ID NO: 202 - protein, 5 aa, artificial sequence
  any amino acid
SSEED

SEQ ID NO: 203 - protein, 5 aa, artificial sequence
  any amino acid
YCSDS

SEQ ID NO: 204 - protein, 5 aa, artificial sequence
  any amino acid
LLMSL

SEQ ID NO: 205 - protein, 5 aa, artificial sequence
  any amino acid
RLVSS

SEQ ID NO: 206 - protein, 5 aa, artificial sequence
  any amino acid
LYQPD

SEQ ID NO: 207 - protein, 5 aa, artificial sequence
  any amino acid
LETLY

SEQ ID NO: 208 - protein, 5 aa, artificial sequence
  any amino acid
TYCTT

SEQ ID NO: 209 - protein, 5 aa, artificial sequence
  any amino acid
SKKTL

SEQ ID NO: 210 - protein, 5 aa, artificial sequence
  any amino acid
LLLLS

SEQ ID NO: 211 - protein, 5 aa, artificial sequence
  any amino acid
IETVY

SEQ ID NO: 212 - protein, 5 aa, artificial sequence
  any amino acid
LETVY

SEQ ID NO: 213 - protein, 5 aa, artificial sequence
  any amino acid
LTRTQ

SEQ ID NO: 214 - protein, 5 aa, artificial sequence
  any amino acid
RQRQR

SEQ ID NO: 215 - protein, 5 aa, artificial sequence
  any amino acid
TDTVY

SEQ ID NO: 216 - protein, 5 aa, artificial sequence
  any amino acid
YCQLQ

SEQ ID NO: 217 - protein, 5 aa, artificial sequence
  any amino acid
ADTVY

SEQ ID NO: 218 - protein, 5 aa, artificial sequence
  any amino acid
ASSTS

SEQ ID NO: 219 - protein, 5 aa, artificial sequence
  any amino acid
DATAT

SEQ ID NO: 220 - protein, 5 aa, artificial sequence
  any amino acid
YTSLQ

SEQ ID NO: 221 - protein, 5 aa, artificial sequence
  any amino acid
SRYYY

SEQ ID NO: 222 - protein, 5 aa, artificial sequence
  any amino acid
TRTAT

SEQ ID NO: 223 - protein, 5 aa, artificial sequence
  any amino acid
KFVRD

SEQ ID NO: 224 - protein, 5 aa, artificial sequence
  any amino acid
SVGTL

SEQ ID NO: 225 - protein, 5 aa, artificial sequence
  any amino acid
EEIEI

SEQ ID NO: 226 - protein, 5 aa, artificial sequence
  any amino acid
QPKPQ

SEQ ID NO: 227 - protein, 5 aa, artificial sequence
  any amino acid
HSRTG

SEQ ID NO: 228 - protein, 5 aa, artificial sequence
  any amino acid
TLMTL

SEQ ID NO: 229 - protein, 5 aa, artificial sequence
  any amino acid
VRTST

SEQ ID NO: 230 - protein, 5 aa, artificial sequence
  any amino acid
VYGAS

SEQ ID NO: 231 - protein, 5 aa, artificial sequence
  any amino acid
LRLSC

SEQ ID NO: 232 - protein, 5 aa, artificial sequence
  any amino acid
RLSCV

SEQ ID NO: 233 - protein, 5 aa, artificial sequence
  any amino acid
RNNWP

SEQ ID NO: 234 - protein, 5 aa, artificial sequence
  any amino acid
YSDSV

SEQ ID NO: 235 - protein, 5 aa, artificial sequence
  any amino acid
YYSDS

SEQ ID NO: 236 - protein, 5 aa, artificial sequence
  any amino acid
AGSYT

SEQ ID NO: 237 - protein, 7 aa, artificial sequence
  any amino acid
  misc_feature (3)..(3): Xaa can be any naturally occurring amino acid
  misc_feature (5)..(5): Xaa can be any naturally occurring amino acid
VWXRXPP

SEQ ID NO: 238 - protein, 9 aa, artificial sequence
  any amino acid
  misc_feature (2)..(3): Xaa can be any naturally occurring amino acid
  misc_feature (5)..(5): Xaa can be any naturally occurring amino acid
  misc_feature (7)..(7): Xaa can be any naturally occurring amino acid
FXXWXRXPP

SEQ ID NO: 239 - protein, 7 aa, artificial sequence
  any amino acid
  misc_feature (3)..(3): Xaa can be any naturally occurring amino acid
  misc_feature (5)..(5): Xaa can be any naturally occurring amino acid
TCXVXGA

SEQ ID NO: 240 - protein, 7 aa, artificial sequence
  any amino acid
  misc_feature (3)..(3): Xaa can be any naturally occurring amino acid
  misc_feature (5)..(5): Xaa can be any naturally occurring amino acid
YSXSXYG

SEQ ID NO: 241 - protein, 7 aa, artificial sequence
  any amino acid
  misc_feature (3)..(3): Xaa can be any naturally occurring amino acid
  misc_feature (5)..(5): Xaa can be any naturally occurring amino acid
YSXSXYG

SEQ ID NO: 242 - protein, 7 aa, artificial sequence
  any amino acid
  misc_feature (3)..(3): Xaa can be any naturally occurring amino acid
  misc_feature (5)..(5): Xaa can be any naturally occurring amino acid
LLXLXLS

SEQ ID NO: 243 - protein, 7 aa, artificial sequence
  any amino acid
  misc_feature (3)..(3): Xaa can be any naturally occurring amino acid
  misc_feature (5)..(5): Xaa can be any naturally occurring amino acid
IEXTXVY

SEQ ID NO: 244 - protein, 7 aa, artificial sequence
  any amino acid
  misc_feature (3)..(3): Xaa can be any naturally occurring amino acid
  misc_feature (5)..(5): Xaa can be any naturally occurring amino acid
RQXRXQR

SEQ ID NO: 245 - protein, 7 aa, artificial sequence
  any amino acid
  misc_feature (3)..(3): Xaa can be any naturally occurring amino acid
  misc_feature (5)..(5): Xaa can be any naturally occurring amino acid
LTXRXTQ

SEQ ID NO: 246 - protein, 7 aa, artificial sequence
  any amino acid
  misc_feature (3)..(3): Xaa can be any naturally occurring amino acid
  misc_feature (5)..(5): Xaa can be any naturally occurring amino acid
LEXTXVY

SEQ ID NO: 247 - protein, 7 aa, artificial sequence
  any amino acid
  misc_feature (3)..(3): Xaa can be any naturally occurring amino acid
  misc_feature (5)..(5): Xaa can be any naturally occurring amino acid
TDXTXVY

SEQ ID NO: 248 - protein, 7 aa, artificial sequence
  any amino acid
  misc_feature (3)..(3): Xaa can be any naturally occurring amino acid
  misc_feature (5)..(5): Xaa can be any naturally occurring amino acid
ADXTXVY

SEQ ID NO: 249 - protein, 7 aa, artificial sequence
  any amino acid
  misc_feature (3)..(3): Xaa can be any naturally occurring amino acid
  misc_feature (5)..(5): Xaa can be any naturally occurring amino acid
YCXQXLQ

SEQ ID NO: 250 - protein, 9 aa, artificial sequence
  any amino acid
  misc_feature (2)..(3): Xaa can be any naturally occurring amino acid
  misc_feature (5)..(5): Xaa can be any naturally occurring amino acid
  misc_feature (7)..(7): Xaa can be any naturally occurring amino acid
LXXVXRXRS

SEQ ID NO: 251 - protein, 9 aa, artificial sequence
  any amino acid
  misc_feature (2)..(3): Xaa can be any naturally occurring amino acid
  misc_feature (5)..(5): Xaa can be any naturally occurring amino acid
  misc_feature (7)..(7): Xaa can be any naturally occurring amino acid
SXXVXGXTL

SEQ ID NO: 252 - protein, 9 aa, artificial sequence
  any amino acid
  misc_feature (2)..(3): Xaa can be any naturally occurring amino acid
  misc_feature (5)..(5): Xaa can be any naturally occurring amino acid
  misc_feature (7)..(7): Xaa can be any naturally occurring amino acid
TXXRXTXAT

SEQ ID NO: 253 - protein, 9 aa, artificial sequence
  any amino acid
  misc_feature (2)..(3): Xaa can be any naturally occurring amino acid
  misc_feature (5)..(5): Xaa can be any naturally occurring amino acid
  misc_feature (7)..(7): Xaa can be any naturally occurring amino acid
SXXRXYXYY

SEQ ID NO: 254 - protein, 9 aa, artificial sequence
  any amino acid
  misc_feature (2)..(3): Xaa can be any naturally occurring amino acid
  misc_feature (5)..(5): Xaa can be any naturally occurring amino acid
  misc_feature (7)..(7): Xaa can be any naturally occurring amino acid
YXXTXSXLQ

SEQ ID NO: 255 - protein, 9 aa, artificial sequence
  any amino acid
  misc_feature (2)..(3): Xaa can be any naturally occurring amino acid
  misc_feature (5)..(5): Xaa can be any naturally occurring amino acid
  misc_feature (7)..(7): Xaa can be any naturally occurring amino acid
KXXFXVXRD

SEQ ID NO: 256 - protein, 9 aa, artificial sequence
  any amino acid
  misc_feature (2)..(3): Xaa can be any naturally occurring amino acid
  misc_feature (5)..(5): Xaa can be any naturally occurring amino acid
  misc_feature (7)..(7): Xaa can be any naturally occurring amino acid
QXXPXKXPQ

SEQ ID NO: 257 - protein, 9 aa, artificial sequence
  any amino acid
  misc_feature (2)..(3): Xaa can be any naturally occurring amino acid
  misc_feature (5)..(5): Xaa can be any naturally occurring amino acid
  misc_feature (7)..(7): Xaa can be any naturally occurring amino acid
EXXEXIXEI

SEQ ID NO: 258 - protein, 9 aa, artificial sequence
  any amino acid
  misc_feature (2)..(3): Xaa can be any naturally occurring amino acid
  misc_feature (5)..(5): Xaa can be any naturally occurring amino acid
  misc_feature (7)..(7): Xaa can be any naturally occurring amino acid
HXXSXRXTG

SEQ ID NO: 259 - protein, 9 aa, artificial sequence
  any amino acid
LIDLRLSCV

SEQ ID NO: 260 - protein, 9 aa, artificial sequence
  any amino acid
IDLRLSCVY

SEQ ID NO: 261 - protein, 9 aa, artificial sequence
  any amino acid
LLDLRLSCV

SEQ ID NO: 262 - protein, 9 aa, artificial sequence
  any amino acid
LDLRLSCVY

SEQ ID NO: 263 - protein, 8 aa, artificial sequence
  any amino acid
  misc_feature (1)..(2): Xaa can be any naturally occurring amino acid
  misc_feature (8)..(8): Xaa can be any naturally occurring amino acid
XXKKSLYX

SEQ ID NO: 264 - protein, 8 aa, artificial sequence
  any amino acid
  misc_feature (1)..(2): Xaa can be any naturally occurring amino acid
  misc_feature (8)..(8): Xaa can be any naturally occurring amino acid
XXVYGASX

SEQ ID NO: 265 - protein, 8 aa, artificial sequence
  any amino acid
  misc_feature (1)..(2): Xaa can be any naturally occurring amino acid
  misc_feature (8)..(8): Xaa can be any naturally occurring amino acid
XXLRLSCX

SEQ ID NO: 266 - protein, 8 aa, artificial sequence
  any amino acid
  misc_feature (1)..(2): Xaa can be any naturally occurring amino acid
  misc_feature (8)..(8): Xaa can be any naturally occurring amino acid
XXRLSCVX

SEQ ID NO: 267 - protein, 8 aa, artificial sequence
  any amino acid
  misc_feature (1)..(2): Xaa can be any naturally occurring amino acid
  misc_feature (8)..(8): Xaa can be any naturally occurring amino acid
XXRNNWPX

SEQ ID NO: 268 - protein, 8 aa, artificial sequence
  any amino acid
  misc_feature (1)..(2): Xaa can be any naturally occurring amino acid
  misc_feature (8)..(8): Xaa can be any naturally occurring amino acid
XXYSDSVX

SEQ ID NO: 269 - protein, 8 aa, artificial sequence
  any amino acid
  misc_feature (1)..(2): Xaa can be any naturally occurring amino acid
  misc_feature (8)..(8): Xaa can be any naturally occurring amino acid
XXYYSDSX

SEQ ID NO: 270 - protein, 8 aa, artificial sequence
  any amino acid
  misc_feature (1)..(2): Xaa can be any naturally occurring amino acid
  misc_feature (8)..(8): Xaa can be any naturally occurring amino acid
XXAGSYTX

SEQ ID NO: 271 - protein, 15 aa, artificial sequence
  any amino acid
LDLQPETTDLYCYEQ

SEQ ID NO: 272 - protein, 15 aa, artificial sequence
  any amino acid
LDLQPEATDLYCYEQ

SEQ ID NO: 273 - protein, 15 aa, artificial sequence
  any amino acid
LDLYPEPTDLYCYEQ

SEQ ID NO: 274 - protein, 7 aa, artificial sequence
  any amino acid
  misc_feature (3)..(3): Xaa can be any naturally occurring amino acid
  misc_feature (5)..(5): Xaa can be any naturally occurring amino acid
SSXEXED

SEQ ID NO: 275 - protein, 7 aa, artificial sequence
  any amino acid
  misc_feature (3)..(3): Xaa can be any naturally occurring amino acid
  misc_feature (5)..(5): Xaa can be any naturally occurring amino acid
PEXTXLY

SEQ ID NO: 276 - protein, 7 aa, artificial sequence
  any amino acid
  misc_feature (3)..(3): Xaa can be any naturally occurring amino acid
  misc_feature (5)..(5): Xaa can be any naturally occurring amino acid
YCXSXDS

SEQ ID NO: 277 - protein, 15 aa, artificial sequence
  any amino acid
EARIELVVESSADDL

SEQ ID NO: 278 - protein, 15 aa, artificial sequence
  any amino acid
IVTCCYTCGTTVRLC

SEQ ID NO: 279 - protein, 9 aa, artificial sequence
  any amino acid
  misc_feature (2)..(3): Xaa can be any naturally occurring amino acid
  misc_feature (5)..(5): Xaa can be any naturally occurring amino acid
  misc_feature (7)..(7): Xaa can be any naturally occurring amino acid
RXXLXVXSS

SEQ ID NO: 280 - protein, 9 aa, artificial sequence
  any amino acid
  misc_feature (2)..(3): Xaa can be any naturally occurring amino acid
  misc_feature (5)..(5): Xaa can be any naturally occurring amino acid
  misc_feature (7)..(7): Xaa can be any naturally occurring amino acid
LXXLXMXSL

SEQ ID NO: 281 - protein, 9 aa, artificial sequence
  any amino acid
  misc_feature (2)..(3): Xaa can be any naturally occurring amino acid
  misc_feature (5)..(5): Xaa can be any naturally occurring amino acid
  misc_feature (7)..(7): Xaa can be any naturally occurring amino acid
LXXYXQXPD

SEQ ID NO: 282 - protein, 9 aa, artificial sequence
  any amino acid
  misc_feature (2)..(3): Xaa can be any naturally occurring amino acid
  misc_feature (5)..(5): Xaa can be any naturally occurring amino acid
  misc_feature (7)..(7): Xaa can be any naturally occurring amino acid
LXXEXTXLY

SEQ ID NO: 283 - protein, 9 aa, artificial sequence
  any amino acid
  misc_feature (2)..(3): Xaa can be any naturally occurring amino acid
  misc_feature (5)..(5): Xaa can be any naturally occurring amino acid
  misc_feature (7)..(7): Xaa can be any naturally occurring amino acid
SXXKXKXTL

SEQ ID NO: 284 - protein, 8 aa, artificial sequence
  any amino acid
  misc_feature (2)..(3): Xaa can be any naturally occurring amino acid
  misc_feature (5)..(5): Xaa can be any naturally occurring amino acid
TXXYXCTT

SEQ ID NO: 285 - protein, 8 aa, artificial sequence
  any amino acid
  misc_feature (1)..(2): Xaa can be any naturally occurring amino acid
  misc_feature (8)..(8): Xaa can be any naturally occurring amino acid
XXSRDTLX

SEQ ID NO: 286 - protein, 5 aa, artificial sequence
  any amino acid
TLTST

SEQ ID NO: 287 - protein, 15 aa, artificial sequence
  any amino acid
SHLTTLATISTSPQP

SEQ ID NO: 288 - protein, 5 aa, artificial sequence
  any amino acid
KLIEA

SEQ ID NO: 289 - protein, 15 aa, artificial sequence
  any amino acid
TPVYKLDISEATQVG

SEQ ID NO: 290 - protein, 5 aa, artificial sequence
  any amino acid
YYTIR

SEQ ID NO: 291 - protein, 15 aa, artificial sequence
  any amino acid
PSSGYYSTTIRYQAT

SEQ ID NO: 292 - protein, 5 aa, artificial sequence
  any amino acid
QFLLN

SEQ ID NO: 293 - protein, 15 aa, artificial sequence
  any amino acid
RFTPQFLLQLNETIY

SEQ ID NO: 294 - protein, 5 aa, artificial sequence
  any amino acid
ATSSP

SEQ ID NO: 295 - protein, 15 aa, artificial sequence
  any amino acid
LTTLATISTSPQPPT

SEQ ID NO: 296 - protein, 5 aa, artificial sequence
  any amino acid
SSDAT

SEQ ID NO: 297 - protein, 15 aa, artificial sequence
  any amino acid
SKSADSLDLATTTSP

SEQ ID NO: 298 - protein, 5 aa, artificial sequence
  any amino acid
RAGGT

SEQ ID NO: 299 - protein, 15 aa, artificial sequence
  any amino acid
TIRYQATGFGTNETE

SEQ ID NO: 300 - protein, 5 aa, artificial sequence
  any amino acid
SYTIR

SEQ ID NO: 301 - protein, 15 aa, artificial sequence
  any amino acid
PSSGYYSTTIRYQAT

SEQ ID NO: 302 - protein, 5 aa, artificial sequence
  any amino acid
VQKNP

SEQ ID NO: 303 - protein, 15 aa, artificial sequence
  any amino acid
VIVNAQPKCNPNLHY

SEQ ID NO: 304 - protein, 5 aa, artificial sequence
  any amino acid
TLTST

SEQ ID NO: 305 - protein, 15 aa, artificial sequence
  any amino acid
SHLTTLATISTSPQS

SEQ ID NO: 306 - protein, 5 aa, artificial sequence
  any amino acid
KLIEA

SEQ ID NO: 307 - protein, 15 aa, artificial sequence
  any amino acid
TPVYKLDISEATQVE

SEQ ID NO: 308 - protein, 5 aa, artificial sequence
  any amino acid
YYTIR

SEQ ID NO: 309 - protein, 15 aa, artificial sequence
  any amino acid
PSSGYYSTTIRYQAT

SEQ ID NO: 310 - protein, 5 aa, artificial sequence
  any amino acid
SKTFL

SEQ ID NO: 311 - protein, 15 aa, artificial sequence
  any amino acid
NTNTSKSTDFLDPAT

SEQ ID NO: 312 - protein, 5 aa, artificial sequence
  any amino acid
QFLLN

SEQ ID NO: 313 - protein, 15 aa, artificial sequence
  any amino acid
RFTPQFLLQLNETIY

SEQ ID NO: 314 - protein, 5 aa, artificial sequence
  any amino acid
ATSSP

SEQ ID NO: 315 - protein, 15 aa, artificial sequence
  any amino acid
LTTLATISTSPQSLT

SEQ ID NO: 316 - protein, 5 aa, artificial sequence
  any amino acid
RAGGT

SEQ ID NO: 317 - protein, 15 aa, artificial sequence
  any amino acid
TIRYQATGFGTNETE

SEQ ID NO: 318 - protein, 5 aa, artificial sequence
  any amino acid
SYTIR

SEQ ID NO: 319 - protein, 15 aa, artificial sequence
  any amino acid
PSSGYYSTTIRYQAT

SEQ ID NO: 320 - protein, 5 aa, artificial sequence
  any amino acid
VQKNP

SEQ ID NO: 321 - protein, 15 aa, artificial sequence
  any amino acid
AIVNAQPKCNPNLHY

SEQ ID NO: 322 - protein, 5 aa, artificial sequence
  any amino acid
SGSDI

SEQ ID NO: 323 - protein, 15 aa, artificial sequence
  any amino acid
PSQNSTEGRRVDVNT

SEQ ID NO: 324 - protein, 5 aa, artificial sequence
  any amino acid
STGRV

SEQ ID NO: 325 - protein, 15 aa, artificial sequence
  any amino acid
NLEGSGVSTDIPSAT

SEQ ID NO: 326 - protein, 5 aa, artificial sequence
  any amino acid
YASLE

SEQ ID NO: 327 - protein, 15 aa, artificial sequence
  any amino acid
GLSSSQILSSSPTMA

SEQ ID NO: 328 - protein, 5 aa, artificial sequence
  any amino acid
SQLSS

SEQ ID NO: 329 - protein, 15 aa, artificial sequence
  any amino acid
TSSYYATSYLEYEIE

SEQ ID NO: 330 - protein, 5 aa, artificial sequence
  any amino acid
TETTI

SEQ ID NO: 331 - protein, 15 aa, artificial sequence
  any amino acid
QETITETTATIIGTN

SEQ ID NO: 332 - protein, 5 aa, artificial sequence
  any amino acid
TTTTT

SEQ ID NO: 333 - protein, 15 aa, artificial sequence
  any amino acid
VNTQETITETTATII

SEQ ID NO: 334 - protein, 5 aa, artificial sequence
  any amino acid
SISSP

SEQ ID NO: 335 - protein, 15 aa, artificial sequence
  any amino acid
LSSSQILSSSPTMAP

SEQ ID NO: 336 - protein, 5 aa, artificial sequence
  any amino acid
SGRDV

SEQ ID NO: 337 - protein, 15 aa, artificial sequence
  any amino acid
QNSTEGRRVDVNTQE

SEQ ID NO: 338 - protein, 5 aa, artificial sequence
  any amino acid
LTGLI

SEQ ID NO: 339 - protein, 15 aa, artificial sequence
  any amino acid
QQLSNTTGKLIWTLD

SEQ ID NO: 340 - protein, 5 aa, artificial sequence
  any amino acid
SPQVS

SEQ ID NO: 341 - protein, 15 aa, artificial sequence
  any amino acid
FRSGVPPQVVSYEAG

SEQ ID NO: 342 - protein, 5 aa, artificial sequence
  any amino acid
LYINR

SEQ ID NO: 343 - protein, 15 aa, artificial sequence
  any amino acid
TELRTYTILNRKAID

SEQ ID NO: 344 - protein, 5 aa, artificial sequence
  any amino acid
VAGGP

SEQ ID NO: 345 - protein, 15 aa, artificial sequence
  any amino acid
RYVHKAQGTGPCPGD

SEQ ID NO: 346 - protein, 30 aa, artificial sequence
  any amino acid
GNGVATDVPSATKRWGFRSGVPPKVVNYEA

SEQ ID NO: 347 - protein, 32 aa, artificial sequence
  any amino acid
HKVSGTGPCAGDFAFHKEGAFFLYDRLASTVI

SEQ ID NO: 348 - protein, 30 aa, artificial sequence
  any amino acid
SGKRSNTTGKLIWKVNPEIDTTIGEWAFWE

SEQ ID NO: 349 - protein, 32 aa, artificial sequence
  any amino acid
AIVNAQPKCNPNLHYWTTQDEGAAIGLAWIPY

SEQ ID NO: 350 - protein, 30 aa, artificial sequence
  any amino acid
WTTQDEGAAIGLAWIPYFGPAAEGIYIEGL

SEQ ID NO: 351 - protein, 31 aa, artificial sequence
  any amino acid
RQLANETTQALQLFLRATTELRTFSILNRKA

SEQ ID NO: 352 - protein, 20 aa, artificial sequence
  any amino acid
PDQGDNDNWWTGWRQWIPAG

SEQ ID NO: 353 - protein, 151 aa, artificial sequence
  any amino acid
VNAQPKCNPNLHYWTTQDEGAAIGLAWIPYFGPAAEGIYIEGLMHNQDGLICGLRQLANETTQALQLFLRATTELRTFSILNRKAIDFLLQRWGGTCHILGPDCCIEPHDWTKNITDKIDQIIHDFVDKTLPDQGDNDNWWTGWRQWIPAG

SEQ ID NO: 354 - protein, 5 aa, artificial sequence
  any amino acid
HPRLR

SEQ ID NO: 355 - protein, 15 aa, artificial sequence
  any amino acid
GIPDHPLRLLRIGNQ

SEQ ID NO: 356 - protein, 5 aa, artificial sequence
  any amino acid
MVVSG

SEQ ID NO: 357 - protein, 15 aa, artificial sequence
  any amino acid
ILEAMVNVISGPKVL

SEQ ID NO: 358 - protein, 5 aa, artificial sequence
  any amino acid
GNALT

SEQ ID NO: 359 - protein, 15 aa, artificial sequence
  any amino acid
SGKKGNSADLTSPEK

SEQ ID NO: 360 - protein, 5 aa, artificial sequence
  any amino acid
DTSGA

SEQ ID NO: 361 - protein, 15 aa, artificial sequence
  any amino acid
TDDTPTGSNGALRPG

SEQ ID NO: 362 - protein, 5 aa, artificial sequence
  any amino acid
SSTAI

SEQ ID NO: 363 - protein, 15 aa, artificial sequence
  any amino acid
TYSFDSTTAAIMLAS

SEQ ID NO: 364 - protein, 5 aa, artificial sequence
  any amino acid
LLLTQ

SEQ ID NO: 365 - protein, 15 aa, artificial sequence
  any amino acid
FDLTALKLITQPLPA

SEQ ID NO: 366 - protein, 5 aa, artificial sequence
  any amino acid
ATGVS

SEQ ID NO: 367 - protein, 15 aa, artificial sequence
  any amino acid
DHASHTPGSVSSAFI

SEQ ID NO: 368 - protein, 5 aa, artificial sequence
  any amino acid
TTTSN

SEQ ID NO: 369 - protein, 15 aa, artificial sequence
  any amino acid
TWTDDTPTGSNGALR

SEQ ID NO: 370 - protein, 5 aa, artificial sequence
  any amino acid
TKTKN

SEQ ID NO: 371 - protein, 15 aa, artificial sequence
  any amino acid
KLTGKKVTSKNGQPI

SEQ ID NO: 372 - protein, 5 aa, artificial sequence
  any amino acid
KNALT

SEQ ID NO: 373 - protein, 15 aa, artificial sequence
  any amino acid
SGKKGNSADLTSPEK

SEQ ID NO: 374 - protein, 5 aa, artificial sequence
  any amino acid
HPRLR

SEQ ID NO: 375 - protein, 15 aa, artificial sequence
  any amino acid
GIPDHPLRLLRIGNQ

SEQ ID NO: 376 - protein, 5 aa, artificial sequence
  any amino acid
MVVSG

SEQ ID NO: 377 - protein, 15 aa, artificial sequence
  any amino acid
ILEAMVNVISGPKVL

SEQ ID NO: 378 - protein, 5 aa, artificial sequence
  any amino acid
GNALT

SEQ ID NO: 379 - protein, 15 aa, artificial sequence
  any amino acid
SGKKGNSADLTSPEK

SEQ ID NO: 380 - protein, 5 aa, artificial sequence
  any amino acid
DTSGA

SEQ ID NO: 381 - protein, 15 aa, artificial sequence
  any amino acid
TDDTPTGSNGALRPG

SEQ ID NO: 382 - protein, 5 aa, artificial sequence
  any amino acid
SSTAI

SEQ ID NO: 383 - protein, 15 aa, artificial sequence
  any amino acid
TYSFDSTTAAIMLAS

SEQ ID NO: 384 - protein, 5 aa, artificial sequence
  any amino acid
LLLTQ

SEQ ID NO: 385 - protein, 15 aa, artificial sequence
  any amino acid
FDLTALKLITQPLPA

SEQ ID NO: 386 - protein, 5 aa, artificial sequence
  any amino acid
ATGVS

SEQ ID NO: 387 - protein, 15 aa, artificial sequence
  any amino acid
DHASHTPGSVSSAFI

SEQ ID NO: 388 - protein, 5 aa, artificial sequence
  any amino acid
TTTSN

SEQ ID NO: 389 - protein, 15 aa, artificial sequence
  any amino acid
TWTDDTPTGSNGALR

SEQ ID NO: 390 - protein, 5 aa, artificial sequence
  any amino acid
TKTKN

SEQ ID NO: 391 - protein, 15 aa, artificial sequence
  any amino acid
KLTGKKVTSKNGQPI

SEQ ID NO: 392 - protein, 5 aa, artificial sequence
  any amino acid
KNALT

SEQ ID NO: 393 - protein, 15 aa, artificial sequence
  any amino acid
SGKKGNSADLTSPEK

SEQ ID NO: 394 - protein, 5 aa, artificial sequence
  any amino acid
SPKLE

SEQ ID NO: 395 - protein, 15 aa, artificial sequence
  any amino acid
YNLISPKKDLEKGVV

SEQ ID NO: 396 - protein, 5 aa, artificial sequence
  any amino acid
SLMSL

SEQ ID NO: 397 - protein, 15 aa, artificial sequence
  any amino acid
KEQLSLKMLSLIRSN

SEQ ID NO: 398 - protein, 5 aa, artificial sequence
  any amino acid
SPKLE

SEQ ID NO: 399 - protein, 15 aa, artificial sequence
  any amino acid
YNLISPKKDLEKGVV

SEQ ID NO: 400 - protein, 5 aa, artificial sequence
  any amino acid
SLMSL

SEQ ID NO: 401 - protein, 15 aa, artificial sequence
  any amino acid
KEQLSLKMLSLIRSN

SEQ ID NO: 402 - protein, 37 aa, artificial sequence
  any amino acid
SHTPGSVSSAFILEAMVNVISGPKVLMKQIPIWLPLG

SEQ ID NO: 403 - protein, 42 aa, artificial sequence
  any amino acid
GKKVTSKNGQPIIPVLLPKYIGLDPVAPGDLTMVITQDCDTC

SEQ ID NO: 404 - protein, 26 aa, artificial sequence
  any amino acid
PNSTIESPLWALRVILAAGIQDQLID

SEQ ID NO: 405 - protein, 434 aa, artificial sequence
  any amino acid
METDTLLLWVLLLWVPGSTGDTRVNAQPKCNPNLHYWTTQDEGAAIGLAWIPYFGPAAEGIYIEGLMHNQDGLICGLRQLANETTQALQLFLRATTELRTFSILNRKAIDFLLQRWGGTCHILGPDCCIEPHDWTKNITDKIDQIIHDFVDKTLPDQGDNDNWWTGWRQWIPAGGGGGSGGGGSGGPGSGGGGSGGGGSASTEPKSCDKTHTCPPCPAPELLGGPSVFLFPPKPKDTLMISRTPEVTCVVVDVSHEDPEVKFNWYVDGVEVHNAKTKPREEQYNSTYRVVSVLTVLHQDWLNGKEYKCKVSNKALPAPIEKTISKAKGQPREPQVYTLPPSREEMTKNQVSLTCLVKGFYPSDIAVEWESNGQPENNYKTTPPVLDSDGSFFLYSKLTVDKSRWQQGNVFSCSVMHEALHNHYTQKSLSLSPGK

SEQ ID NO: 406 - protein, 434 aa, artificial sequence
  any amino acid
METDTLLLWVLLLWVPGSTGDTRVNAQPKCNPNLHYWTTQDEGAAIGLAWIPYFGPAAEGIYIEGLMHNQDGLICGLRQLANETTQALQLFLRATTELRTFSILNRKAIDFLLQRWGGTCHILGPDCCIEPHDWTKNITDKIDQIIHDFVDKTLPDQGDNDNWWTGWRQWIPAGGGGGSGGGGSGGPGSGGGGSGGGGSVDEPRGPTIKPCPPCKCPAPNLLGGPSVFIFPPKIKDVLMISLSPIVTCVVVDVSEDDPDVQISWFVNNVEVHTAQTQTHREDYNSTLRVVSALPIQHQDWMSGKEFKCKVNNKDLPAPIERTISKPKGSVRAPQVYVLPPPEEEMTKKQVTLTCMVTDFMPEDIYVEWTNNGKTELNYKNTEPVLDSDGSYFMYSKLRVEKKNWVERNSYSCSVVHEGLHNHHTTKSFSRTPGK

SEQ ID NO: 407 - protein, 313 aa, artificial sequence
  any amino acid
METDTLLLWVLLLWVPGSTGDTRGNGVATDVPSATKRWGFRSGVPPKVVNYEAGGGGSGGGGSGGPGSGGGGSGGGGSASTEPKSCDKTHTCPPCPAPELLGGPSVFLFPPKPKDTLMISRTPEVTCVVVDVSHEDPEVKFNWYVDGVEVHNAKTKPREEQYNSTYRVVSVLTVLHQDWLNGKEYKCKVSNKALPAPIEKTISKAKGQPREPQVYTLPPSREEMTKNQVSLTCLVKGFYPSDIAVEWESNGQPENNYKTTPPVLDSDGSFFLYSKLTVDKSRWQQGNVFSCSVMHEALHNHYTQKSLSLSPGK

SEQ ID NO: 408 - protein, 313 aa, artificial sequence
  any amino acid
METDTLLLWVLLLWVPGSTGDTRGNGVATDVPSATKRWGFRSGVPPKVVNYEAGGGGSGGGGSGGPGSGGGGSGGGGSVDEPRGPTIKPCPPCKCPAPNLLGGPSVFIFPPKIKDVLMISLSPIVTCVVVDVSEDDPDVQISWFVNNVEVHTAQTQTHREDYNSTLRVVSALPIQHQDWMSGKEFKCKVNNKDLPAPIERTISKPKGSVRAPQVYVLPPPEEEMTKKQVTLTCMVTDFMPEDIYVEWTNNGKTELNYKNTEPVLDSDGSYFMYSKLRVEKKNWVERNSYSCSVVHEGLHNHHTTKSFSRTPGK

SEQ ID NO: 409 - protein, 315 aa, artificial sequence
  any amino acid
METDTLLLWVLLLWVPGSTGDTRHKVSGTGPCAGDFAFHKEGAFFLYDRLASTVIGGGGSGGGGSGGPGSGGGGSGGGGSASTEPKSCDKTHTCPPCPAPELLGGPSVFLFPPKPKDTLMISRTPEVTCVVVDVSHEDPEVKFNWYVDGVEVHNAKTKPREEQYNSTYRVVSVLTVLHQDWLNGKEYKCKVSNKALPAPIEKTISKAKGQPREPQVYTLPPSREEMTKNQVSLTCLVKGFYPSDIAVEWESNGQPENNYKTTPPVLDSDGSFFLYSKLTVDKSRWQQGNVFSCSVMHEALHNHYTQKSLSLSPGK

SEQ ID NO: 410 - protein, 314 aa, artificial sequence
  any amino acid
METDTLLLWVLLLWVPGSTGDTRHKVSGTGPCAGDFAFHKEGAFFLYDRLASTVIGGGGSGGGGSGGPGSGGGGSGGGGSVDEPRGPTIKPCPPCKCPAPNLLGGPSVFIFPPKIKDVLMISLSPIVTCVVVDVSEDDPDVQISWFVNNVEVHTAQTQTHREDYNSTLRVVSALPIQHQDWMSGKEFKCKVNNKDLPAPIERTISKPKGSVRAPQVYVLPPPEEEMTKKQVTLTCMVTDFMPEDIYVEWTNNGKTELNYKNTEPVLDSDGSYFMYSKLRVEKKNWVERNSYSCSVVHEGLHNHHTTKSFSRTPG

SEQ ID NO: 411 - protein, 313 aa, artificial sequence
  any amino acid
METDTLLLWVLLLWVPGSTGDTRSGKRSNTTGKLIWKVNPEIDTTIGEWAFWEGGGGSGGGGSGGPGSGGGGSGGGGSASTEPKSCDKTHTCPPCPAPELLGGPSVFLFPPKPKDTLMISRTPEVTCVVVDVSHEDPEVKFNWYVDGVEVHNAKTKPREEQYNSTYRVVSVLTVLHQDWLNGKEYKCKVSNKALPAPIEKTISKAKGQPREPQVYTLPPSREEMTKNQVSLTCLVKGFYPSDIAVEWESNGQPENNYKTTPPVLDSDGSFFLYSKLTVDKSRWQQGNVFSCSVMHEALHNHYTQKSLSLSPGK

SEQ ID NO: 412 - protein, 313 aa, artificial sequence
  any amino acid
METDTLLLWVLLLWVPGSTGDTRSGKRSNTTGKLIWKVNPEIDTTIGEWAFWEGGGGSGGGGSGGPGSGGGGSGGGGSVDEPRGPTIKPCPPCKCPAPNLLGGPSVFIFPPKIKDVLMISLSPIVTCVVVDVSEDDPDVQISWFVNNVEVHTAQTQTHREDYNSTLRVVSALPIQHQDWMSGKEFKCKVNNKDLPAPIERTISKPKGSVRAPQVYVLPPPEEEMTKKQVTLTCMVTDFMPEDIYVEWTNNGKTELNYKNTEPVLDSDGSYFMYSKLRVEKKNWVERNSYSCSVVHEGLHNHHTTKSFSRTPGK

SEQ ID NO: 413 - protein, 315 aa, artificial sequence
  any amino acid
METDTLLLWVLLLWVPGSTGDTRAIVNAQPKCNPNLHYWTTQDEGAAIGLAWIPYGGGGSGGGGSGGPGSGGGGSGGGGSASTEPKSCDKTHTCPPCPAPELLGGPSVFLFPPKPKDTLMISRTPEVTCVVVDVSHEDPEVKFNWYVDGVEVHNAKTKPREEQYNSTYRVVSVLTVLHQDWLNGKEYKCKVSNKALPAPIEKTISKAKGQPREPQVYTLPPSREEMTKNQVSLTCLVKGFYPSDIAVEWESNGQPENNYKTTPPVLDSDGSFFLYSKLTVDKSRWQQGNVFSCSVMHEALHNHYTQKSLSLSPGK

SEQ ID NO: 414 - protein, 315 aa, artificial sequence
  any amino acid
METDTLLLWVLLLWVPGSTGDTRAIVNAQPKCNPNLHYWTTQDEGAAIGLAWIPYGGGGSGGGGSGGPGSGGGGSGGGGSVDEPRGPTIKPCPPCKCPAPNLLGGPSVFIFPPKIKDVLMISLSPIVTCVVVDVSEDDPDVQISWFVNNVEVHTAQTQTHREDYNSTLRVVSALPIQHQDWMSGKEFKCKVNNKDLPAPIERTISKPKGSVRAPQVYVLPPPEEEMTKKQVTLTCMVTDFMPEDIYVEWTNNGKTELNYKNTEPVLDSDGSYFMYSKLRVEKKNWVERNSYSCSVVHEGLHNHHTTKSFSRTPGK

SEQ ID NO: 415 - protein, 313 aa, artificial sequence
  any amino acid
METDTLLLWVLLLWVPGSTGDTRWTTQDEGAAIGLAWIPYFGPAAEGIYIEGLGGGGSGGGGSGGPGSGGGGSGGGGSASTEPKSCDKTHTCPPCPAPELLGGPSVFLFPPKPKDTLMISRTPEVTCVVVDVSHEDPEVKFNWYVDGVEVHNAKTKPREEQYNSTYRVVSVLTVLHQDWLNGKEYKCKVSNKALPAPIEKTISKAKGQPREPQVYTLPPSREEMTKNQVSLTCLVKGFYPSDIAVEWESNGQPENNYKTTPPVLDSDGSFFLYSKLTVDKSRWQQGNVFSCSVMHEALHNHYTQKSLSLSPGK

SEQ ID NO: 416 - protein, 313 aa, artificial sequence
  any amino acid
METDTLLLWVLLLWVPGSTGDTRWTTQDEGAAIGLAWIPYFGPAAEGIYIEGLGGGGSGGGGSGGPGSGGGGSGGGGSVDEPRGPTIKPCPPCKCPAPNLLGGPSVFIFPPKIKDVLMISLSPIVTCVVVDVSEDDPDVQISWFVNNVEVHTAQTQTHREDYNSTLRVVSALPIQHQDWMSGKEFKCKVNNKDLPAPIERTISKPKGSVRAPQVYVLPPPEEEMTKKQVTLTCMVTDFMPEDIYVEWTNNGKTELNYKNTEPVLDSDGSYFMYSKLRVEKKNWVERNSYSCSVVHEGLHNHHTTKSFSRTPGK

SEQ ID NO: 417 - protein, 314 aa, artificial sequence
  any amino acid
METDTLLLWVLLLWVPGSTGDTRRQLANETTQALQLFLRATTELRTFSILNRKAGGGGSGGGGSGGPGSGGGGSGGGGSASTEPKSCDKTHTCPPCPAPELLGGPSVFLFPPKPKDTLMISRTPEVTCVVVDVSHEDPEVKFNWYVDGVEVHNAKTKPREEQYNSTYRVVSVLTVLHQDWLNGKEYKCKVSNKALPAPIEKTISKAKGQPREPQVYTLPPSREEMTKNQVSLTCLVKGFYPSDIAVEWESNGQPENNYKTTPPVLDSDGSFFLYSKLTVDKSRWQQGNVFSCSVMHEALHNHYTQKSLSLSPGK

SEQ ID NO: 418 - protein, 314 aa, artificial sequence
  any amino acid
METDTLLLWVLLLWVPGSTGDTRRQLANETTQALQLFLRATTELRTFSILNRKAGGGGSGGGGSGGPGSGGGGSGGGGSVDEPRGPTIKPCPPCKCPAPNLLGGPSVFIFPPKIKDVLMISLSPIVTCVVVDVSEDDPDVQISWFVNNVEVHTAQTQTHREDYNSTLRVVSALPIQHQDWMSGKEFKCKVNNKDLPAPIERTISKPKGSVRAPQVYVLPPPEEEMTKKQVTLTCMVTDFMPEDIYVEWTNNGKTELNYKNTEPVLDSDGSYFMYSKLRVEKKNWVERNSYSCSVVHEGLHNHHTTKSFSRTPGK

SEQ ID NO: 419 - protein, 303 aa, artificial sequence
  any amino acid
METDTLLLWVLLLWVPGSTGDTRPDQGDNDNWWTGWRQWIPAGGGGGSGGGGSGGPGSGGGGSGGGGSASTEPKSCDKTHTCPPCPAPELLGGPSVFLFPPKPKDTLMISRTPEVTCVVVDVSHEDPEVKFNWYVDGVEVHNAKTKPREEQYNSTYRVVSVLTVLHQDWLNGKEYKCKVSNKALPAPIEKTISKAKGQPREPQVYTLPPSREEMTKNQVSLTCLVKGFYPSDIAVEWESNGQPENNYKTTPPVLDSDGSFFLYSKLTVDKSRWQQGNVFSCSVMHEALHNHYTQKSLSLSPGK

SEQ ID NO: 420 - protein, 303 aa, artificial sequence
  any amino acid
METDTLLLWVLLLWVPGSTGDTRPDQGDNDNWWTGWRQWIPAGGGGGSGGGGSGGPGSGGGGSGGGGSVDEPRGPTIKPCPPCKCPAPNLLGGPSVFIFPPKIKDVLMISLSPIVTCVVVDVSEDDPDVQISWFVNNVEVHTAQTQTHREDYNSTLRVVSALPIQHQDWMSGKEFKCKVNNKDLPAPIERTISKPKGSVRAPQVYVLPPPEEEMTKKQVTLTCMVTDFMPEDIYVEWTNNGKTELNYKNTEPVLDSDGSYFMYSKLRVEKKNWVERNSYSCSVVHEGLHNHHTTKSFSRTPGK

SEQ ID NO: 421 - protein, 320 aa, artificial sequence
  any amino acid
METDTLLLWVLLLWVPGSTGDTRSHTPGSVSSAFILEAMVNVISGPKVLMKQIPIWLPLGGGGGSGGGGSGGPGSGGGGSGGGGSASTEPKSCDKTHTCPPCPAPELLGGPSVFLFPPKPKDTLMISRTPEVTCVVVDVSHEDPEVKFNWYVDGVEVHNAKTKPREEQYNSTYRVVSVLTVLHQDWLNGKEYKCKVSNKALPAPIEKTISKAKGQPREPQVYTLPPSREEMTKNQVSLTCLVKGFYPSDIAVEWESNGQPENNYKTTPPVLDSDGSFFLYSKLTVDKSRWQQGNVFSCSVMHEALHNHYTQKSLSLSPGK

SEQ ID NO: 422 - protein, 320 aa, artificial sequence
  any amino acid
METDTLLLWVLLLWVPGSTGDTRSHTPGSVSSAFILEAMVNVISGPKVLMKQIPIWLPLGGGGGSGGGGSGGPGSGGGGSGGGGSVDEPRGPTIKPCPPCKCPAPNLLGGPSVFIFPPKIKDVLMISLSPIVTCVVVDVSEDDPDVQISWFVNNVEVHTAQTQTHREDYNSTLRVVSALPIQHQDWMSGKEFKCKVNNKDLPAPIERTISKPKGSVRAPQVYVLPPPEEEMTKKQVTLTCMVTDFMPEDIYVEWTNNGKTELNYKNTEPVLDSDGSYFMYSKLRVEKKNWVERNSYSCSVVHEGLHNHHTTKSFSRTPGK

SEQ ID NO: 423 - protein, 325 aa, artificial sequence
  any amino acid
METDTLLLWVLLLWVPGSTGDTRGKKVTSKNGQPIIPVLLPKYIGLDPVAPGDLTMVITQDCDTCGGGGSGGGGSGGPGSGGGGSGGGGSASTEPKSCDKTHTCPPCPAPELLGGPSVFLFPPKPKDTLMISRTPEVTCVVVDVSHEDPEVKFNWYVDGVEVHNAKTKPREEQYNSTYRVVSVLTVLHQDWLNGKEYKCKVSNKALPAPIEKTISKAKGQPREPQVYTLPPSREEMTKNQVSLTCLVKGFYPSDIAVEWESNGQPENNYKTTPPVLDSDGSFFLYSKLTVDKSRWQQGNVFSCSVMHEALHNHYTQKSLSLSPGK

SEQ ID NO: 424 - protein, 325 aa, artificial sequence
  any amino acid
METDTLLLWVLLLWVPGSTGDTRGKKVTSKNGQPIIPVLLPKYIGLDPVAPGDLTMVITQDCDTCGGGGSGGGGSGGPGSGGGGSGGGGSVDEPRGPTIKPCPPCKCPAPNLLGGPSVFIFPPKIKDVLMISLSPIVTCVVVDVSEDDPDVQISWFVNNVEVHTAQTQTHREDYNSTLRVVSALPIQHQDWMSGKEFKCKVNNKDLPAPIERTISKPKGSVRAPQVYVLPPPEEEMTKKQVTLTCMVTDFMPEDIYVEWTNNGKTELNYKNTEPVLDSDGSYFMYSKLRVEKKNWVERNSYSCSVVHEGLHNHHTTKSFSRTPGK

SEQ ID NO: 425 - protein, 309 aa, artificial sequence
  any amino acid
METDTLLLWVLLLWVPGSTGDTRPNSTIESPLWALRVILAAGIQDQLIDGGGGSGGGGSGGPGSGGGGSGGGGSASTEPKSCDKTHTCPPCPAPELLGGPSVFLFPPKPKDTLMISRTPEVTCVVVDVSHEDPEVKFNWYVDGVEVHNAKTKPREEQYNSTYRVVSVLTVLHQDWLNGKEYKCKVSNKALPAPIEKTISKAKGQPREPQVYTLPPSREEMTKNQVSLTCLVKGFYPSDIAVEWESNGQPENNYKTTPPVLDSDGSFFLYSKLTVDKSRWQQGNVFSCSVMHEALHNHYTQKSLSLSPGK

SEQ ID NO: 426 - protein, 309 aa, artificial sequence
  any amino acid
METDTLLLWVLLLWVPGSTGDTRPNSTIESPLWALRVILAAGIQDQLIDGGGGSGGGGSGGPGSGGGGSGGGGSVDEPRGPTIKPCPPCKCPAPNLLGGPSVFIFPPKIKDVLMISLSPIVTCVVVDVSEDDPDVQISWFVNNVEVHTAQTQTHREDYNSTLRVVSALPIQHQDWMSGKEFKCKVNNKDLPAPIERTISKPKGSVRAPQVYVLPPPEEEMTKKQVTLTCMVTDFMPEDIYVEWTNNGKTELNYKNTEPVLDSDGSYFMYSKLRVEKKNWVERNSYSCSVVHEGLHNHHTTKSFSRTPGK

SEQ ID NO: 427 - protein, 504 aa, artificial sequence
  any amino acid
METDTLLLWVLLLWVPGSTGDTRVNAQPKCNPNLHYWTTQDEGAAIGLAWIPYFGPAAEGIYIEGLMHNQDGLICGLRQLANETTQALQLFLRATTELRTFSILNRKAIDFLLQRWGGTCHILGPDCCIEPHDWTKNITDKIDQIIHDFVDKTLPDQGDNDNWWTGWRQWIPAGASTKGPSVFPLAPSSKSTSGGTAALGCLVKDYFPEPVTVSWNSGALTSGVHTFPAVLQSSGLYSLSSVVTVPSSSLGTQTYICNVNHKPSNTKVDKRVEPKSCDKTHTCPPCPAPELLGGPSVFLFPPKPKDTLMISRTPEVTCVVVDVSHEDPEVKFNWYVDGVEVHNAKTKPREEQYNSTYRVVSVLTVLHQDWLNGKEYKCKVSNKALPAPIEKTISKAKGQPREPQVYTLPPSREEMTKNQVSLTCLVKGFYPSDIAVEWESNGQPENNYKTTPPVLDSDGSFFLYSKLTVDKSRWQQGNVFSCSVMHEALHNHYTQKSLSLSPGK

SEQ ID NO: 428 - protein, 280 aa, artificial sequence
  any amino acid
METDTLLLWVLLLWVPGSTGDTRVNAQPKCNPNLHYWTTQDEGAAIGLAWIPYFGPAAEGIYIEGLMHNQDGLICGLRQLANETTQALQLFLRATTELRTFSILNRKAIDFLLQRWGGTCHILGPDCCIEPHDWTKNITDKIDQIIHDFVDKTLPDQGDNDNWWTGWRQWIPAGTVAAPSVFIFPPSDEQLKSGTASVVCLLNNFYPREAKVQWKVDNALQSGNSQESVTEQDSKDSTYSLSSTLTLSKADYEKHKVYACEVTHQGLSSPVTKSFNRGEC

SEQ ID NO: 429 - protein, 504 aa, artificial sequence
  any amino acid
METDTLLLWVLLLWVPGSTGDTRVNAQPKCNPNLHYWTTQDEGAAIGLAWIPYFGPAAEGIYIEGLMHNQDGLICGLRQLANETTQALQLFLRATTELRTFSILNRKAIDFLLQRWGGTCHILGPDCCIEPHDWTKNITDKIDQIIHDFVDKTLPDQGDNDNWWTGWRQWIPAGAKTTAPSVYPLAPVCGDTTGSSVTLGCLVKGYFPEPVTLTWNSGSLSSGVHTFPAVLQSDLYTLSSSVTVTSSTWPSQSITCNVAHPASSTKVDKKIEPRGPTIKPCPPCKCPAPNLLGGPSVFIFPPKIKDVLMISLSPIVTCVVVDVSEDDPDVQISWFVNNVEVHTAQTQTHREDYNSTLRVVSALPIQHQDWMSGKEFKCKVNNKDLPAPIERTISKPKGSVRAPQVYVLPPPEEEMTKKQVTLTCMVTDFMPEDIYVEWTNNGKTELNYKNTEPVLDSDGSYFMYSKLRVEKKNWVERNSYSCSVVHEGLHNHHTTKSFSRTPGK

SEQ ID NO: 430 - protein, 282 aa, artificial sequence
  any amino acid
METDTLLLWVLLLWVPGSTGDTRVNAQPKCNPNLHYWTTQDEGAAIGLAWIPYFGPAAEGIYIEGLMHNQDGLICGLRQLANETTQALQLFLRATTELRTFSILNRKAIDFLLQRWGGTCHILGPDCCIEPHDWTKNITDKIDQIIHDFVDKTLPDQGDNDNWWTGWRQWIPAGKRADAAPTVSIFPPSSEQLTSGGASVVCFLNNFYPKDINVKWKIDGSERQNGVLNSWTDQDSKDSTYSMSSTLTLTKDEYERHNSYTCEATHKTSTSPIVKSFNRNEC

SEQ ID NO: 431 - protein, 816 aa, artificial sequence
  any amino acid
METDTLLLWVLLLWVPGSTGDTRVNAQPKCNPNLHYWTTQDEGAAIGLAWIPYFGPAAEGIYIEGLMHNQDGLICGLRQLANETTQALQLFLRATTELRTFSILNRKAIDFLLQRWGGTCHILGPDCCIEPHDWTKNITDKIDQIIHDFVDKTLPDQGDNDNWWTGWRQWIPAGGGGGSVNAQPKCNPNLHYWTTQDEGAAIGLAWIPYFGPAAEGIYIEGLMHNQDGLICGLRQLANETTQALQLFLRATTELRTFSILNRKAIDFLLQRWGGTCHILGPDCCIEPHDWTKNITDKIDQIIHDFVDKTLPDQGDNDNWWTGWRQWIPAGGGGGSVNAQPKCNPNLHYWTTQDEGAAIGLAWIPYFGPAAEGIYIEGLMHNQDGLICGLRQLANETTQALQLFLRATTELRTFSILNRKAIDFLLQRWGGTCHILGPDCCIEPHDWTKNITDKIDQIIHDFVDKTLPDQGDNDNWWTGWRQWIPAGASTKGPSVFPLAPSSKSTSGGTAALGCLVKDYFPEPVTVSWNSGALTSGVHTFPAVLQSSGLYSLSSVVTVPSSSLGTQTYICNVNHKPSNTKVDKRVEPKSCDKTHTCPPCPAPELLGGPSVFLFPPKPKDTLMISRTPEVTCVVVDVSHEDPEVKFNWYVDGVEVHNAKTKPREEQYNSTYRVVSVLTVLHQDWLNGKEYKCKVSNKALPAPIEKTISKAKGQPREPQVYTLPPSREEMTKNQVSLTCLVKGFYPSDIAVEWESNGQPENNYKTTPPVLDSDGSFFLYSKLTVDKSRWQQGNVFSCSVMHEALHNHYTQKSLSLSPGK

SEQ ID NO: 432 - protein, 816 aa, artificial sequence
  any amino acid
METDTLLLWVLLLWVPGSTGDTRVNAQPKCNPNLHYWTTQDEGAAIGLAWIPYFGPAAEGIYIEGLMHNQDGLICGLRQLANETTQALQLFLRATTELRTFSILNRKAIDFLLQRWGGTCHILGPDCCIEPHDWTKNITDKIDQIIHDFVDKTLPDQGDNDNWWTGWRQWIPAGGGGGSVNAQPKCNPNLHYWTTQDEGAAIGLAWIPYFGPAAEGIYIEGLMHNQDGLICGLRQLANETTQALQLFLRATTELRTFSILNRKAIDFLLQRWGGTCHILGPDCCIEPHDWTKNITDKIDQIIHDFVDKTLPDQGDNDNWWTGWRQWIPAGGGGGSVNAQPKCNPNLHYWTTQDEGAAIGLAWIPYFGPAAEGIYIEGLMHNQDGLICGLRQLANETTQALQLFLRATTELRTFSILNRKAIDFLLQRWGGTCHILGPDCCIEPHDWTKNITDKIDQIIHDFVDKTLPDQGDNDNWWTGWRQWIPAGAKTTAPSVYPLAPVCGDTTGSSVTLGCLVKGYFPEPVTLTWNSGSLSSGVHTFPAVLQSDLYTLSSSVTVTSSTWPSQSITCNVAHPASSTKVDKKIEPRGPTIKPCPPCKCPAPNLLGGPSVFIFPPKIKDVLMISLSPIVTCVVVDVSEDDPDVQISWFVNNVEVHTAQTQTHREDYNSTLRVVSALPIQHQDWMSGKEFKCKVNNKDLPAPIERTISKPKGSVRAPQVYVLPPPEEEMTKKQVTLTCMVTDFMPEDIYVEWTNNGKTELNYKNTEPVLDSDGSYFMYSKLRVEKKNWVERNSYSCSVVHEGLHNHHTTKSFSRTPGK

SEQ ID NO: 433 - protein, 856 aa, artificial sequence
  any amino acid
METDTLLLWVLLLWVPGSTGDTRVNAQPKCNPNLHYWTTQDEGAAIGLAWIPYFGPAAEGIYIEGLMHNQDGLICGLRQLANETTQALQLFLRATTELRTFSILNRKAIDFLLQRWGGTCHILGPDCCIEPHDWTKNITDKIDQIIHDFVDKTLPDQGDNDNWWTGWRQWIPAGGGGGSGGGGSGGPGSGGGGSGGGGSVNAQPKCNPNLHYWTTQDEGAAIGLAWIPYFGPAAEGIYIEGLMHNQDGLICGLRQLANETTQALQLFLRATTELRTFSILNRKAIDFLLQRWGGTCHILGPDCCIEPHDWTKNITDKIDQIIHDFVDKTLPDQGDNDNWWTGWRQWIPAGGGGGSGGGGSGGPGSGGGGSGGGGSVNAQPKCNPNLHYWTTQDEGAAIGLAWIPYFGPAAEGIYIEGLMHNQDGLICGLRQLANETTQALQLFLRATTELRTFSILNRKAIDFLLQRWGGTCHILGPDCCIEPHDWTKNITDKIDQIIHDFVDKTLPDQGDNDNWWTGWRQWIPAGASTKGPSVFPLAPSSKSTSGGTAALGCLVKDYFPEPVTVSWNSGALTSGVHTFPAVLQSSGLYSLSSVVTVPSSSLGTQTYICNVNHKPSNTKVDKRVEPKSCDKTHTCPPCPAPELLGGPSVFLFPPKPKDTLMISRTPEVTCVVVDVSHEDPEVKFNWYVDGVEVHNAKTKPREEQYNSTYRVVSVLTVLHQDWLNGKEYKCKVSNKALPAPIEKTISKAKGQPREPQVYTLPPSREEMTKNQVSLTCLVKGFYPSDIAVEWESNGQPENNYKTTPPVLDSDGSFFLYSKLTVDKSRWQQGNVFSCSVMHEALHNHYTQKSLSLSPGK

SEQ ID NO: 434 - protein, 856 aa, artificial sequence
  any amino acid
METDTLLLWVLLLWVPGSTGDTRVNAQPKCNPNLHYWTTQDEGAAIGLAWIPYFGPAAEGIYIEGLMHNQDGLICGLRQLANETTQALQLFLRATTELRTFSILNRKAIDFLLQRWGGTCHILGPDCCIEPHDWTKNITDKIDQIIHDFVDKTLPDQGDNDNWWTGWRQWIPAGGGGGSGGGGSGGPGSGGGGSGGGGSVNAQPKCNPNLHYWTTQDEGAAIGLAWIPYFGPAAEGIYIEGLMHNQDGLICGLRQLANETTQALQLFLRATTELRTFSILNRKAIDFLLQRWGGTCHILGPDCCIEPHDWTKNITDKIDQIIHDFVDKTLPDQGDNDNWWTGWRQWIPAGGGGGSGGGGSGGPGSGGGGSGGGGSVNAQPKCNPNLHYWTTQDEGAAIGLAWIPYFGPAAEGIYIEGLMHNQDGLICGLRQLANETTQALQLFLRATTELRTFSILNRKAIDFLLQRWGGTCHILGPDCCIEPHDWTKNITDKIDQIIHDFVDKTLPDQGDNDNWWTGWRQWIPAGAKTTAPSVYPLAPVCGDTTGSSVTLGCLVKGYFPEPVTLTWNSGSLSSGVHTFPAVLQSDLYTLSSSVTVTSSTWPSQSITCNVAHPASSTKVDKKIEPRGPTIKPCPPCKCPAPNLLGGPSVFIFPPKIKDVLMISLSPIVTCVVVDVSEDDPDVQISWFVNNVEVHTAQTQTHREDYNSTLRVVSALPIQHQDWMSGKEFKCKVNNKDLPAPIERTISKPKGSVRAPQVYVLPPPEEEMTKKQVTLTCMVTDFMPEDIYVEWTNNGKTELNYKNTEPVLDSDGSYFMYSKLRVEKKNWVERNSYSCSVVHEGLHNHHTTKSFSRTPGK

SEQ ID NO: 435 - DNA, 75 bp, artificial sequence
  any amino acid
ggtggtggcggttcaggcggaggtggctctggcggtcccggatccggcggaggtggctctggcggaggagggtct

SEQ ID NO: 436 - protein, 25 aa, artificial sequence
  any amino acid
GGGGSGGGGSGGPGSGGGGSGGGGS

SEQ ID NO: 437 - protein, 15 aa, artificial sequence
  any amino acid
RWLYPESTVLYFTFH

SEQ ID NO: 438 - protein, 15 aa, artificial sequence
  any amino acid
LFLMPEMTFLYGAII

SEQ ID NO: 439 - protein, 15 aa, artificial sequence
  any amino acid
DDLWPELTSLYVVFT

SEQ ID NO: 440 - protein, 15 aa, artificial sequence
  any amino acid
IQLLPEGTVLYVCPT

SEQ ID NO: 441 - protein, 15 aa, artificial sequence
  any amino acid
MSLMPELTGLYISYV

SEQ ID NO: 442 - protein, 15 aa, artificial sequence
  any amino acid
LLLFPEATNLYTIEK

SEQ ID NO: 443 - protein, 15 aa, artificial sequence
  any amino acid
NAGSGIIISDTPVHD

SEQ ID NO: 444 - protein, 15 aa, artificial sequence
  any amino acid
FVLFPEATKLYLHGV

SEQ ID NO: 445 - protein, 15 aa, artificial sequence
  any amino acid
KRLYPESTLLYVSLC

SEQ ID NO: 446 - protein, 15 aa, artificial sequence
  any amino acid
LELLPEGTLLYVCPI

SEQ ID NO: 447 - protein, 15 aa, artificial sequence
  any amino acid
RWLYPESTVLYFTFH

SEQ ID NO: 448 - protein, 15 aa, artificial sequence
  any amino acid
LQLVPEGTALYLYEL

SEQ ID NO: 449 - protein, 15 aa, artificial sequence
  any amino acid
FWLQPEYTALYAMLD

SEQ ID NO: 450 - protein, 15 aa, artificial sequence
  any amino acid
LQLMPEGTLLYVCPG

SEQ ID NO: 451 - protein, 15 aa, artificial sequence
  any amino acid
QMLLPELTVLYPGCA

SEQ ID NO: 452 - protein, 15 aa, artificial sequence
  any amino acid
LLLKPECTSLYSMLI

SEQ ID NO: 453 - protein, 15 aa, artificial sequence
  any amino acid
LSLLPEITALYMLIQ

SEQ ID NO: 454 - protein, 15 aa, artificial sequence
  any amino acid
IVLVPEITQLYLRLC

SEQ ID NO: 455 - protein, 15 aa, artificial sequence
  any amino acid
MLLNPEGTVLYTCAQ

SEQ ID NO: 456 - protein, 15 aa, artificial sequence
  any amino acid
CHLCPETTRLYIHST

SEQ ID NO: 457 - protein, 15 aa, artificial sequence
  any amino acid
LLLGPEGTVLYICSQ

SEQ ID NO: 458 - protein, 15 aa, artificial sequence
  any amino acid
ICLRPECTQLYKRHV

SEQ ID NO: 459 - protein, 15 aa, artificial sequence
  any amino acid
CCLCPETTRLYVQST

SEQ ID NO: 460 - protein, 15 aa, artificial sequence
  any amino acid
CHLCPETTRLYIHST

SEQ ID NO: 461 - protein, 15 aa, artificial sequence
  any amino acid
LLLGPEGTVLYNCST

SEQ ID NO: 462 - protein, 15 aa, artificial sequence
  any amino acid
LHLEPEDTFLYEQLC

SEQ ID NO: 463 - protein, 15 aa, artificial sequence
  any amino acid
CHLCPETTRLYIHST

SEQ ID NO: 464 - protein, 15 aa, artificial sequence
  any amino acid
CCLCPETTRLYVQST

SEQ ID NO: 465 - protein, 15 aa, artificial sequence
  any amino acid
RCLKPEDTGLYRDIV

SEQ ID NO: 466 - protein, 97 aa, artificial sequence
  any amino acid
MRGHKPTLKEYVLDLYPEPTDLYCYEQLSDSSDEDEGLDRPDGQAQPATADYYIVTCCHTCNTTVRLCVNSTASDLRTIQQLLMGTVNIVCPTCAQQ

SEQ ID NO: 467 - DNA, 1611 bp, artificial sequence
  any amino acid
atggccataagtggagtccctgtgctaggatttttcatcatagctgtgctgatgagcgctcaggaatcatgggctatcaaagaagaacatgtgatcatccaggccgagttctatctgaatcctgaccaatcaggcgagtttatgtttgactttgatggtgatgagattttccatgtggatatggcaaagaaggagacggtctggcggcttgaagaatttggacgatttgccagctttgaggctcaaggtgcattggccaacatagctgtggacaaagccaacctggaaatcatgacaaagcgctccaactatactccgatcaccaatgtacctccagaggtaactgtgctcacgaacagccctgtggaactgagagagcccaacgtcctcatctgtttcatcgacaagttcaccccaccagtggtcaatgtcacgtggcttcgaaatggaaaacctgtcaccacaggagtgtcagagacagtcttcctgcccagggaagaccaccttttccgcaagttccactatctccccttcctgccctcaactgaggacgtttacgactgcagggtggagcactggggcttggatgagcctcttctcaagcactgggagtttgatgtgtcgaccaagggcccatcggtcttccccctggcaccctctagcaagagcacctctgggggcacagcggccctgggctgcctggtcaaggactacttccccgaaccggtgacggtgtcgtggaactcaggcgccctgaccagcggcgtgcacaccttcccggctgtcctacagtcctcaggactctactccctcagcagcgtggtgaccgtgccctccagcagcttgggcacccagacctacatctgcaacgtgaatcacaagcccagcaacaccaaggtggacaagagagttgagcccaaatcttgtgacaaaactcacacatgcccaccgtgcccagcacctgaactcctggggggaccgtcagtcttcctcttccccccaaaacccaaggacaccctcatgatctcccggacccctgaggtcacatgcgtggtggtggacgtgagccacgaagaccctgaggtcaagttcaactggtacgtggacggcgtggaggtgcataatgccaagacaaagccgcgggaggagcagtacaacagcacgtaccgtgtggtcagcgtcctcaccgtcctgcaccaggactggctgaatggcaaggagtacaagtgcaaggtctccaacaaagccctcccagcccccatcgagaaaaccatctccaaagccaaagggcagccccgagaaccacaggtgtacaccctgcccccatcccgggaggagatgaccaagaaccaggtcagcctgacctgcctggtcaaaggcttctatcccagcgacatcgccgtggagtgggagagcaatgggcagccggagaacaactacaagaccacgcctcccgtgctggactccgacggctccttcttcctctatagcaagctcaccgtggacaagagcaggtggcagcaggggaacgtcttctcatgctccgtgatgcatgaggctctgcacaaccactacacgcagaagagcctctccctgtctccgggtaaatga

SEQ ID NO: 468 - protein, 536 aa, artificial sequence
  any amino acid
MAISGVPVLGFFIIAVLMSAQESWAIKEEHVIIQAEFYLNPDQSGEFMFDFDGDEIFHVDMAKKETVWRLEEFGRFASFEAQGALANIAVDKANLEIMTKRSNYTPITNVPPEVTVLTNSPVELREPNVLICFIDKFTPPVVNVTWLRNGKPVTTGVSETVFLPREDHLFRKFHYLPFLPSTEDVYDCRVEHWGLDEPLLKHWEFDVSTKGPSVFPLAPSSKSTSGGTAALGCLVKDYFPEPVTVSWNSGALTSGVHTFPAVLQSSGLYSLSSVVTVPSSSLGTQTYICNVNHKPSNTKVDKRVEPKSCDKTHTCPPCPAPELLGGPSVFLFPPKPKDTLMISRTPEVTCVVVDVSHEDPEVKFNWYVDGVEVHNAKTKPREEQYNSTYRVVSVLTVLHQDWLNGKEYKCKVSNKALPAPIEKTISKAKGQPREPQVYTLPPSREEMTKNQVSLTCLVKGFYPSDIAVEWESNGQPENNYKTTPPVLDSDGSFFLYSKLTVDKSRWQQGNVFSCSVMHEALHNHYTQKSLSLSPGK

SEQ ID NO: 469 - protein, 5 aa, artificial sequence
  any amino acid
GSYAD

SEQ ID NO: 470 - protein, 5 aa, artificial sequence
  any amino acid
AGGII

SEQ ID NO: 471 - protein, 5 aa, artificial sequence
  any amino acid
NASII

SEQ ID NO: 472 - protein, 5 aa, artificial sequence
  any amino acid
SVSVS

SEQ ID NO: 473 - protein, 5 aa, artificial sequence
  any amino acid
PGQAP

SEQ ID NO: 474 - protein, 9 aa, artificial sequence
  any amino acid
AAGIGILTV

SEQ ID NO: 475 - protein, 15 aa, artificial sequence
  any amino acid
LGVLLLIGCWYCRRR

SEQ ID NO: 476 - protein, 7 aa, artificial sequence
  any amino acid
  misc_feature (3)..(3): Xaa can be any naturally occurring amino acid
  misc_feature (5)..(5): Xaa can be any naturally occurring amino acid
LLXGXWY

SEQ ID NO: 477 - protein, 15 aa, artificial sequence
  any amino acid
LGVLLLIGCWYCRRR

SEQ ID NO: 478 - protein, 9 aa, artificial sequence
  any amino acid
  misc_feature (2)..(3): Xaa can be any naturally occurring amino acid
  misc_feature (5)..(5): Xaa can be any naturally occurring amino acid
  misc_feature (7)..(7): Xaa can be any naturally occurring amino acid
VXXLXGXWY

SEQ ID NO: 479 - protein, 15 aa, artificial sequence
  any amino acid
VSFGVWIRTPPAYRP

SEQ ID NO: 480 - protein, 5 aa, artificial sequence
  any amino acid
FWRPP

SEQ ID NO: 481 - protein, 5 aa, artificial sequence
  any amino acid
VWRPP

SEQ ID NO: 482 - protein, 15 aa, artificial sequence
  any amino acid
VSFGVWIRTPPAYRP

SEQ ID NO: 483 - protein, 5 aa, artificial sequence
  any amino acid
FWRPP

SEQ ID NO: 484 - protein, 5 aa, artificial sequence
  any amino acid
VWRPP

SEQ ID NO: 485 - protein, 5 aa, artificial sequence
  any amino acid
VQKNP

SEQ ID NO: 486 - protein, 5 aa, artificial sequence
  any amino acid
GGGGS

SEQ ID NO: 487 - protein, 5 aa, artificial sequence
  any amino acid
PETLY

SEQ ID NO: 488 - protein, 5 aa, artificial sequence
  any amino acid
LETLY